European Patent Specification EP 3 609 911 B1, published July 5, 2023. Title: Multivalent OspA polypeptides and methods and uses relating thereto. Applicant: Valneva Austria GmbH. The sequence listing filed with the application follows.

SEQUENCE LISTING (75 sequences)

SEQ ID NO: 1 - protein, 268 aa, Artificial Sequence
  Artificial sequence
  LIPID (1)..(1)
CSSFKQNVSSLDEKNSVSVDLPGEMKVLVSKEKNKDGKYDLIATVDKLELKGTSDKNNGSGVLEGVKADKSKVKLTISDDLGQTTLEVFKEDGKTLVSKKVTSKDKSSTEEKFNEKGEVSEKIITRADGTRLEYTGIKSDGSGKAKEVLKGYVLEGTLTAEKTTLVVKEGTVTLSKNISKSGEVSVELNDTDSSAATKKTAAWNSGTSTLTITVNSKKTKDLVFTKENTITVQQYDSNGTKLEGSAVEITKLDEIKNALKLEHHHHHH

SEQ ID NO: 2 - protein, 268 aa, Artificial Sequence
  Artificial sequence
  LIPID (1)..(1)
CSSFKQNVSSLDEKNSASVDLPGEMKVLVSKEKDKDGKYSLKATVDKIELKGTSDKDNGSGVLEGTKDDKSKAKLTIADDLSKTTFELFKEDGKTLVSRKVSSKDKTSTDEMFNEKGELSAKTMTRENGTKLEYTEMKSDGTGKAKEVLKNFTLEGKVANDKVTLEVKEGTVTLSKEIAKSGEVTVALNDTNTTQATKKTGAWDSKTSTLTISVNSKKTTQLVFTKQDTITVQKYDSAGTNLEGTAVEIKTLDELKNALKLEHHHHHH

SEQ ID NO: 3 - protein, 269 aa, Artificial Sequence
  Artificial sequence
  LIPID (1)..(1)
CSSFKQNVSSLDEKNSVSVDLPGGMKVLVSKEKDKDGKYSLMATVEKLELKGTSDKSNGSGVLEGEKADKSKAKLTISQDLNQTTFEIFKEDGKTLVSRKVNSKDKSSTEEKFNDKGKLSEKVVTRANGTRLEYTEIKNDGSGKAKEVLKGFALEGTLTDGGETKLTVTEGTVTLSKNISKSGEITVALNDTETTPADKKTGEWKSDTSTLTISKNSQKTKQLVFTKENTITVQNYNRAGNALEGSPAEIKDLAELKAALKLEHHHHHH

SEQ ID NO: 4 - protein, 268 aa, Artificial Sequence
  Artificial sequence
  LIPID (1)..(1)
CSSFKQNVSSLDEKNSVSVDLPGEMKVLVSKEKDKDGKYSLMATVDKLELKGTSDKSNGSGTLEGEKSDKSKAKLTISEDLSKTTFEIFKEDGKTLVSKKVNSKDKSSIEEKFNAKGELSEKTILRANGTRLEYTEIKSDGTGKAKEVLKDFALEGTLAADKTTLKVTEGTVVLSKHIPNSGEITVELNDSNSTQATKKTGKWDSNTSTLTISVNSKKTKNIVFTKEDTITVQKYDSAGTNLEGNAVEIKTLDELKNALKLEHHHHHH

SEQ ID NO: 5 - protein, 268 aa, Artificial Sequence
  Artificial sequence
  LIPID (1)..(1)
CSSFKQNVSSLDEKNSVSVDLPGGMKVLVSKEKDKDGKYSLMATVEKLELKGTSDKNNGSGTLEGEKTDKSKVKLTIAEDLSKTTFEIFKEDGKTLVSKKVTLKDKSSTEEKFNEKGEISEKTIVRANGTRLEYTDIKSDKTGKAKEVLKDFTLEGTLAADGKTTLKVTEGTVTLSKNISKSGEITVALDDTDSSGNKKSGTWDSGTSTLTISKNRTKTKQLVFTKEDTITVQNYDSAGTNLEGKAVEITTLKELKNALKLEHHHHHH

SEQ ID NO: 6 - protein, 269 aa, Artificial Sequence
  Artificial sequence
  LIPID (1)..(1)
CSSFKQNVSSLDEKNSVSVDLPGGMTVLVSKEKDKDGKYSLEATVDKLELKGTSDKNNGSGTLEGEKTDKSKVKSTIADDLSQTKFEIFKEDGKTLVSKKVTLKDKSSTEEKFNGKGETSEKTIVRANGTRLEYTDIKSDGSGKAKEVLKDFTLEGTLAADGKTTLKVTEGTVVLSKNILKSGEITAALDDSDTTRATKKTGKWDSKTSTLTISVNSQKTKNLVFTKEDTITVQRYDSAGTNLEGKAVEITTLKELKNALKLEHHHHHH

SEQ ID NO: 7 - protein, 148 aa, Borrelia afzelii
FNEKGELSAKTMTRENGTKLEYTEMKSDGTGKAKEVLKNFTLEGKVANDKVTLEVKEGTVTLSKEIAKSGEVTVALNDTNTTQATKKTGAWDSKTSTLTISVNSKKTTQLVFTQKDTITVKQYDSAGTNLEGTAVEIKTLDELKNALK

SEQ ID NO: 8 - protein, 148 aa, Artificial Sequence
  Artificial sequence
FNEKGEISEKTIVRANGTRLEYTDIKSDKTGKAKEVLKDFTLEGTVAADKVTLKVTEGTVTLSKHIPNSGEITVELDDTDSSAATKKTAAWDSNTSTLTITVNSKKTKNLVFTKEDTICVQNYDSNGTNLEGKCVEITTLKELKNALK

SEQ ID NO: 9 - protein, 148 aa, Artificial Sequence
  Artificial sequence
FNEKGEISEKTIVRANGTRLEYTDIKSDKTGKAKEVLKDFTLEGTVAADKVTLKVTCGTVTLSKHIPNSGEITVELDDTDSSAATKKTAAWDSNTSTLTITVNSKKTKNLVFTKEDTITVQNYDSNGTNLEGKAVEITTLKELCNALK

SEQ ID NO: 10 - protein, 149 aa, Artificial Sequence
  Artificial sequence
FNAKGELSEKTILRANGTRLEYTEIKSDGTGKAKEVLKDFALEGTVAADGKVTLKVTCGTVTLSKNISKSGEITVALDDTDSSAATKKTAAWDSGTSTLTITVNSKKTKQLVFTKEDTITVQNYDSNGTNLEGKAVEITTLKELCNALK

SEQ ID NO: 11 - protein, 149 aa, Artificial Sequence
  Artificial sequence
FNAKGELSEKTILRANGTRLEYTEIKSDGTGKAKEVLKDFALEGTVAADGKVTLKVTEGTVTLSKNISKSGEITVALDDTDSSAATKKTAAWDSGTSTLTITVNSKKTKQLVFTKEDTICVQNYDSNGTNLEGKCVEITTLKELKNALK

SEQ ID NO: 12 - protein, 148 aa, Artificial Sequence
  Artificial sequence
FNEKGELSAKTMTRENGTKLEYTEMKSDGTGKAKEVLKNFTLEGKVANDKVTLEVKCGTVTLSKEIAKSGEVTVALNDTNTTRATKKTGKWDSKTSTLTISVNSQKTKNLVFTKEDTITVQNYDSAGTNLEGSPAEIKDLAELCAALK

SEQ ID NO: 13 - protein, 148 aa, Artificial Sequence
  Artificial sequence
FNEKGELSAKTMTRENGTKLEYTEMKSDGTGKAKEVLKNFTLEGKVANDKVTLEVKCGTVTLSKEIAKSGEVTVALNDTNTTQATKKTGAWDSKTSTLTISVNSKKTKNLVFTKEDTITVQNYDSAGTNLEGSPAEIKDLAELCAALK

SEQ ID NO: 14 - protein, 157 aa, Artificial Sequence
  Artificial sequence
  LIPID (1)..(1)
CSSFNEKGEISEKTIVRANGTRLEYTDIKSDKTGKAKEVLKDFTLEGTVAADKVTLKVTEGTVTLSKHIPNSGEITVELDDTDSSAATKKTAAWDSNTSTLTITVNSKKTKNLVFTKEDTICVQNYDSNGTNLEGKCVEITTLKELKNALKHHHHHH

SEQ ID NO: 15 - protein, 157 aa, Artificial Sequence
  Artificial sequence
  LIPID (1)..(1)
CSSFNEKGEISEKTIVRANGTRLEYTDIKSDKTGKAKEVLKDFTLEGTVAADKVTLKVTCGTVTLSKHIPNSGEITVELDDTDSSAATKKTAAWDSNTSTLTITVNSKKTKNLVFTKEDTITVQNYDSNGTNLEGKAVEITTLKELCNALKHHHHHH

SEQ ID NO: 16 - protein, 158 aa, Artificial Sequence
  Artificial sequence
  LIPID (1)..(1)
CSSFNAKGELSEKTILRANGTRLEYTEIKSDGTGKAKEVLKDFALEGTVAADGKVTLKVTCGTVTLSKNISKSGEITVALDDTDSSAATKKTAAWDSGTSTLTITVNSKKTKQLVFTKEDTITVQNYDSNGTNLEGKAVEITTLKELCNALKHHHHHH

SEQ ID NO: 17 - protein, 158 aa, Artificial Sequence
  Artificial sequence
  LIPID (1)..(1)
CSSFNAKGELSEKTILRANGTRLEYTEIKSDGTGKAKEVLKDFALEGTVAADGKVTLKVTEGTVTLSKNISKSGEITVALDDTDSSAATKKTAAWDSGTSTLTITVNSKKTKQLVFTKEDTICVQNYDSNGTNLEGKCVEITTLKELKNALKHHHHHH

SEQ ID NO: 18 - protein, 157 aa, Artificial Sequence
  Artificial sequence
  LIPID (1)..(1)
CSSFNEKGELSAKTMTRENGTKLEYTEMKSDGTGKAKEVLKNFTLEGKVANDKVTLEVKCGTVTLSKEIAKSGEVTVALNDTNTTRATKKTGKWDSKTSTLTISVNSQKTKNLVFTKEDTITVQNYDSAGTNLEGSPAEIKDLAELCAALKHHHHHH

SEQ ID NO: 19 - protein, 157 aa, Artificial Sequence
  Artificial sequence
  LIPID (1)..(1)
CSSFNEKGELSAKTMTRENGTKLEYTEMKSDGTGKAKEVLKNFTLEGKVANDKVTLEVKCGTVTLSKEIAKSGEVTVALNDTNTTQATKKTGAWDSKTSTLTISVNSKKTKNLVFTKEDTITVQNYDSAGTNLEGSPAEIKDLAELCAALKHHHHHH

SEQ ID NO: 20 - protein, 151 aa, Artificial Sequence
  Artificial sequence
  LIPID (1)..(1)
CSSFNEKGEISEKTIVRANGTRLEYTDIKSDKTGKAKEVLKDFTLEGTVAADKVTLKVTEGTVTLSKHIPNSGEITVELDDTDSSAATKKTAAWDSNTSTLTITVNSKKTKNLVFTKEDTICVQNYDSNGTNLEGKCVEITTLKELKNALK

SEQ ID NO: 21 - protein, 151 aa, Artificial Sequence
  Artificial sequence
  LIPID (1)..(1)
CSSFNEKGEISEKTIVRANGTRLEYTDIKSDKTGKAKEVLKDFTLEGTVAADKVTLKVTCGTVTLSKHIPNSGEITVELDDTDSSAATKKTAAWDSNTSTLTITVNSKKTKNLVFTKEDTITVQNYDSNGTNLEGKAVEITTLKELCNALK

SEQ ID NO: 22 - protein, 152 aa, Artificial Sequence
  Artificial sequence
  LIPID (1)..(1)
CSSFNAKGELSEKTILRANGTRLEYTEIKSDGTGKAKEVLKDFALEGTVAADGKVTLKVTCGTVTLSKNISKSGEITVALDDTDSSAATKKTAAWDSGTSTLTITVNSKKTKQLVFTKEDTITVQNYDSNGTNLEGKAVEITTLKELCNALK

SEQ ID NO: 23 - protein, 152 aa, Artificial Sequence
  Artificial sequence
  LIPID (1)..(1)
CSSFNAKGELSEKTILRANGTRLEYTEIKSDGTGKAKEVLKDFALEGTVAADGKVTLKVTEGTVTLSKNISKSGEITVALDDTDSSAATKKTAAWDSGTSTLTITVNSKKTKQLVFTKEDTICVQNYDSNGTNLEGKCVEITTLKELKNALK

SEQ ID NO: 24 - protein, 151 aa, Artificial Sequence
  Artificial sequence
  LIPID (1)..(1)
CSSFNEKGELSAKTMTRENGTKLEYTEMKSDGTGKAKEVLKNFTLEGKVANDKVTLEVKCGTVTLSKEIAKSGEVTVALNDTNTTRATKKTGKWDSKTSTLTISVNSQKTKNLVFTKEDTITVQNYDSAGTNLEGSPAEIKDLAELCAALK

SEQ ID NO: 25 - protein, 151 aa, Artificial Sequence
  Artificial sequence
  LIPID (1)..(1)
CSSFNEKGELSAKTMTRENGTKLEYTEMKSDGTGKAKEVLKNFTLEGKVANDKVTLEVKCGTVTLSKEIAKSGEVTVALNDTNTTQATKKTGAWDSKTSTLTISVNSKKTKNLVFTKEDTITVQNYDSAGTNLEGSPAEIKDLAELCAALK

SEQ ID NO: 26 - protein, 337 aa, Artificial Sequence
  Artificial sequence
  LIPID (1)..(1)
CSSFNAKGELSEKTILRANGTRLEYTEIKSDGTGKAKEVLKDFALEGTVAADGKVTLKVTCGTVTLSKNISKSGEITVALDDTDSSAATKKTAAWDSGTSTLTITVNSKKTKQLVFTKEDTITVQNYDSNGTNLEGKAVEITTLKELCNALKGTSANNQAGQKSSGSTQATTPNLTFEKYSFNEKGELSAKTMTRENGTKLEYTEMKSDGTGKAKEVLKNFTLEGKVANDKVTLEVKCGTVTLSKEIAKSGEVTVALNDTNTTRATKKTGKWDSKTSTLTISVNSQKTKNLVFTKEDTITVQNYDSAGTNLEGSPAEIKDLAELCAALKLEHHHHHH

SEQ ID NO: 27 - DNA, 1011 bp, Artificial Sequence
  Artificial sequence
tgctcaagcttcaatgcaaaaggtgaactgagcgaaaaaaccattctgcgtgcaaatggcacccgtctggaatataccgaaatcaaaagtgatggcaccggtaaagcaaaagaagtgctgaaagattttgcactggaaggcaccgttgcagcagatggtaaagttaccctgaaagttacctgtggcaccgtgaccctgagcaaaaacattagcaaaagcggtgaaattaccgttgccctggatgataccgatagcagcgcagcaaccaaaaaaaccgcagcatgggatagcggcaccagcaccctgaccattaccgttaatagtaaaaaaaccaaacagctggtgtttaccaaagaggataccattacggttcagaactatgatagcaatggtacgaatctggaaggtaaagccgttgaaatcaccacactgaaagaactgtgtaatgcactgaaaggtactagtgcaaataatcaggcaggtcagaaaagcagcggtagcacccaggcaaccaccccgaatctgacctttgaaaagtactcatttaacgagaaaggcgagctgtcagcaaaaaccatgacccgtgaaaatggaaccaaactggaatacacggaaatgaaatcagatggtacaggcaaagccaaagaggtcctgaaaaacttcaccctggaagggaaagttgccaatgataaagtgacactggaagttaaatgtggtacagttacactgagcaaagaaattgccaaatcaggtgaagtgaccgtggcactgaatgatacaaataccacccgtgccacaaaaaaaacaggtaaatgggatagtaaaacgagcacactgacaattagtgtgaatagccagaaaacgaaaaacctggtgttcacgaaagaagatacaatcaccgtacagaattatgattcagcaggcaccaacctggaaggttcaccggcagaaattaaagatctggccgaactgtgtgcagccctgaaactcgagcaccaccaccaccaccac

SEQ ID NO: 28 - protein, 329 aa, Artificial Sequence
  Artificial sequence
  LIPID (1)..(1)
CSSFNAKGELSEKTILRANGTRLEYTEIKSDGTGKAKEVLKDFALEGTVAADGKVTLKVTCGTVTLSKNISKSGEITVALDDTDSSAATKKTAAWDSGTSTLTITVNSKKTKQLVFTKEDTITVQNYDSNGTNLEGKAVEITTLKELCNALKGTSANNQAGQKSSGSTQATTPNLTFEKYSFNEKGELSAKTMTRENGTKLEYTEMKSDGTGKAKEVLKNFTLEGKVANDKVTLEVKCGTVTLSKEIAKSGEVTVALNDTNTTRATKKTGKWDSKTSTLTISVNSQKTKNLVFTKEDTITVQNYDSAGTNLEGSPAEIKDLAELCAALK

SEQ ID NO: 29 - DNA, 987 bp, Artificial Sequence
  Artificial sequence
tgctcaagcttcaatgcaaaaggtgaactgagcgaaaaaaccattctgcgtgcaaatggcacccgtctggaatataccgaaatcaaaagtgatggcaccggtaaagcaaaagaagtgctgaaagattttgcactggaaggcaccgttgcagcagatggtaaagttaccctgaaagttacctgtggcaccgtgaccctgagcaaaaacattagcaaaagcggtgaaattaccgttgccctggatgataccgatagcagcgcagcaaccaaaaaaaccgcagcatgggatagcggcaccagcaccctgaccattaccgttaatagtaaaaaaaccaaacagctggtgtttaccaaagaggataccattacggttcagaactatgatagcaatggtacgaatctggaaggtaaagccgttgaaatcaccacactgaaagaactgtgtaatgcactgaaaggtactagtgcaaataatcaggcaggtcagaaaagcagcggtagcacccaggcaaccaccccgaatctgacctttgaaaagtactcatttaacgagaaaggcgagctgtcagcaaaaaccatgacccgtgaaaatggaaccaaactggaatacacggaaatgaaatcagatggtacaggcaaagccaaagaggtcctgaaaaacttcaccctggaagggaaagttgccaatgataaagtgacactggaagttaaatgtggtacagttacactgagcaaagaaattgccaaatcaggtgaagtgaccgtggcactgaatgatacaaataccacccgtgccacaaaaaaaacaggtaaatgggatagtaaaacgagcacactgacaattagtgtgaatagccagaaaacgaaaaacctggtgttcacgaaagaagatacaatcaccgtacagaattatgattcagcaggcaccaacctggaaggttcaccggcagaaattaaagatctggccgaactgtgtgcagccctgaaa

SEQ ID NO: 30 - protein, 23 aa, Artificial Sequence
  Artificial sequence
MKATKLVLGAVILGSTLLAGCSS

SEQ ID NO: 31 - protein, 6 aa, Artificial Sequence
  Artificial sequence
HHHHHH

SEQ ID NO: 32 - protein, 23 aa, Artificial Sequence
  Artificial sequence
ANNQAGQKSSGSTQATTPNLTFE

SEQ ID NO: 33 - protein, 159 aa, Artificial Sequence
  Artificial sequence
  LIPID (1)..(1)
CSSFNEKGEVSEKIITRADGTRLEYTGIKSDGSGKAKEVLKNFTLEGKVANDKTTLVVKCGTVTLSKNISKSGEVSVELNDTDSSAATKKTAAWNSGTSTLTITVNSKKTKDLVFTKENTITVQQYDSNGTKLEGSAVEITKLDEICNALKLEHHHHHH

SEQ ID NO: 34 - protein, 162 aa, Artificial Sequence
  Artificial sequence
  LIPID (1)..(1)
LIPCSSFNEKGELSAKTMTRENGTKLEYTEMKSDGTGKAKEVLKNFTLEGKVANDKVTLEVKCGTVTLSKEIAKSGEVTVALNDTNTTQATKKTGAWDSKTSTLTISVNSKKTTQLVFTKQDTITVQKYDSAGTNLEGTAVEIKTLDELCNALKLEHHHHHH

SEQ ID NO: 35 - protein, 160 aa, Artificial Sequence
  Artificial sequence
  LIPID (1)..(1)
CSSFNDKGKLSEKVVTRANGTRLEYTEIKNDGSGKAKEVLKGFALEGTLTDGGETKLTVTCGTVTLSKNISKSGEITVALNDTETTPADKKTGEWKSDTSTLTISKNSQKPKQLVFTKENTITVQNYNRAGNALEGSPAEIKDLAELCAALKLEHHHHHH

SEQ ID NO: 36 - protein, 159 aa, Artificial Sequence
  Artificial sequence
  LIPID (1)..(1)
CSSFNAKGELSEKTILRANGTRLEYTEIKSDGTGKAKEVLKDFALEGTLAADKTTLKVTCGTVVLSKHIPNSGEITVELNDSNSTQATKKTGKWDSNTSTLTISVNSKKTKNIVFTKEDTITVQKYDSAGTNLEGNAVEIKTLDELCNALKLEHHHHHH

SEQ ID NO: 37 - protein, 159 aa, Artificial Sequence
  Artificial sequence
  LIPID (1)..(1)
CSSFNEKGEISEKTIVRANGTRLEYTDIKSDKTGKAKEVLKDFTLEGTLAADGKTTLKVTCGTVTLSKNISKSGEITVALDDTDSSGNKKSGTWDSGTSTLTISKNRTKTKQLVFTKEDTITVQNYDSAGTNLEGKAVEITTLKELCNALKLEHHHHHH

SEQ ID NO: 38 - protein, 160 aa, Artificial Sequence
  Artificial sequence
  LIPID (1)..(1)
CSSFNGKGETSEKTIVRANGTRLEYTDIKSDGSGKAKEVLKDFTLEGTLAADGKTTLKVTCGTVVLSKNILKSGEITAALDDSDTTRATKKTGKWDSKTSTLTISVNSQKTKNLVFTKEDTITVQRYDSAGTNLEGKAVEITTLKELCNALKLEHHHHHH

SEQ ID NO: 39 - protein, 11 aa, Artificial Sequence
  Artificial sequence
KLKLLLLLKLK

SEQ ID NO: 40 - DNA, 26 bp, Artificial Sequence
  Artificial sequence
  misc_feature (1)..(26): n=deoxyinosine
ncncncncncncncncncncncncnc

SEQ ID NO: 41 - protein, 150 aa, Artificial Sequence
  Artificial sequence
FNEKGEVSEKILTRSNGTTLEYSQMTDAENATKAVETLKNGIKLPGNLVGGKTKLTVTCGTVTLSKNISKSGEITVALNDTETTPADKKTGEWKSDTSTLTISKNSQKTKQLVFTKENTITVQNYNRAGNALEGSPAEIKDLAELCAALK

SEQ ID NO: 42 - protein, 52 aa, Borrelia valaisiana
FNEKGEVSEKILTRSNGTTLEYSQMTDAENATKAVETLKNGIKLPGNLVGGK

SEQ ID NO: 43 - protein, 98 aa, Borrelia garinii
TKLTVTCGTVTLSKNISKSGEITVALNDTETTPADKKTGEWKSDTSTLTISKNSQKTKQLVFTKENTITVQNYNRAGNALEGSPAEIKDLAELCAALK

SEQ ID NO: 44 - protein, 274 aa, Borrelia valaisiana
MKKYLLGIGLILALIACKQNVSSLDEKNSASVDLPGEMKVLVSKEKDKDGKYSLVATVDKVELKGTSDKNNGSGTLEGVKDDKSKVKLTISDDLGETKLETFKEDGTLVSRKVNFKDKSFTEEKFNEKGEVSEKILTRSNGTTLEYSQMTDAENATKAVETLKNGIKLPGNLVGGKTTLKITEGTVTLSKHIAKSGEVTVEINDTSSTPNTKKTGKWDARNSTLTIIVDSKNKTKLVFTKQDTITVQSYNPAGNKLEGTAVEIKTLQELKNALK

SEQ ID NO: 45 - protein, 273 aa, Borrelia spielmanii
MKKYLLGIGLILALIACKQNVSGLDEKNSTSVDVPGELKVLVSKEKDKDGKYSLMATVDKLELKGTSDKNDGSGVLEGVKADKSKVKLTISDHLSKTTFEVFKEDGKTLVSRNVNSKDKSSTKEKFNEKGELSEKTLVRANGTKLEYTEIKSDGTGKAKEVLKDFTLEGTLANEKATLTVKEGTVTLSKNIDKSGEVTVALNDTDSTAATKKTGAWDSKTSTLTITVNSKKTKDLVFTKQDTITVQKYDSAGTTLEGSAVEIKTLDELKNALK

SEQ ID NO: 46 - protein, 274 aa, Borrelia garinii
MKKYLLGIGLILALIACKQNVSSLDEKNSVSVDLPGGMKVLVSKEKDKDGKYSLMATVEKLELKGTSDKSNGSGVLEGEKADKSKAKLTISQDLNQTTFEIFKEDGKTLVSRKVNSKDKSSTEEKFNDKGKLSEKVVTRANGTRLEYTEIKNDGSGKAKEVLKGFALEGTLTDGGETKLTVTEGTVTLSKNISKSGEITVALNDTETTPADKKTGEWKSDTSTLTISKNSQKTKQLVFTKENTITVQNYNRAGNALEGSPAEIKDLAELKAALK

SEQ ID NO: 47 - DNA, 1029 bp, Artificial Sequence
  Artificial sequence
atgaaagctactaaactggtactgggcgcggtaatcctgggttctactctgctggcaggttgctcaagcttcaatgctaagggcgaactgagcgaaaaaacgatcctgcgtgcgaatggcacccgtctggaatacaccgaaatcaaatccgatggtacgggcaaagcaaaggaagtcctgaaagattttgctctggaaggtaccctggcggccgacaaaaccacgctgaaggtgacgtgcggcaccgtggttctgagcaaacatattccgaactctggtgaaatcaccgttgaactgaacgatagcaattctacgcaggcaaccaaaaagacgggcaaatgggacagtaatacctccacgctgaccatttcagtcaactcgaaaaagaccaaaaatattgtgttcacgaaggaagatacgatcaccgttcaaaaatatgactccgcgggcaccaacctggaaggcaatgccgtcgaaatcaaaaccctggatgaactgtgtaacgccctgaagggtactagtgacaaaaacaatggctctggtagcaaagagaaaaacaaagatggcaagtactcattcaacgaaaaaggcgaagtgagcgaaaaaattctgacccgtagcaatggcaccaccctggaatatagccagatgaccgatgcagaaaatgcaaccaaagcagttgaaaccctgaaaaacggtattaaactgcctggtaatctggttggtggtaaaaccaaactgaccgttacctgtggcaccgttaccctgagcaaaaacattagcaaaagcggtgaaattaccgtggcactgaatgataccgaaaccacaccggcagacaaaaaaaccggtgaatggaaaagcgataccagcaccctgaccattagtaaaaatagccagaaaacaaaacagctggtgtttaccaaagaaaacaccattaccgtgcagaattataaccgtgcaggtaatgcactggaaggtagtccggcagaaattaaagatctggcagaactgtgtgcagccctgaaataa

SEQ ID NO: 48 - protein, 322 aa, Artificial Sequence
  Artificial sequence
  LIPID (1)..(1)
CSSFNAKGELSEKTILRANGTRLEYTEIKSDGTGKAKEVLKDFALEGTLAADKTTLKVTCGTVVLSKHIPNSGEITVELNDSNSTQATKKTGKWDSNTSTLTISVNSKKTKNIVFTKEDTITVQKYDSAGTNLEGNAVEIKTLDELCNALKGTSDKNNGSGSKEKNKDGKYSFNEKGEVSEKILTRSNGTTLEYSQMTDAENATKAVETLKNGIKLPGNLVGGKTKLTVTCGTVTLSKNISKSGEITVALNDTETTPADKKTGEWKSDTSTLTISKNSQKTKQLVFTKENTITVQNYNRAGNALEGSPAEIKDLAELCAALK

SEQ ID NO: 49 - DNA, 1020 bp, Artificial Sequence
  Artificial sequence
atgaaagctactaaactggtactgggcgcggtaatcctgggttctactctgctggcaggttgctcaagcttcaacgaaaagggcgaagtcagcgaaaaaatcattacccgcgcagacggcacccgcctggaatacaccggcatcaaatcggacggcagcggcaaagcgaaagaagttctgaaaaactttaccctggaaggcaaagtcgcaaatgataaaaccaccctggtggtgaaatgcggcaccgttacgctgagcaaaaacattagtaaatccggtgaagtctctgtggaactgaatgataccgacagctctgcggccaccaagaaaaccgcagcttggaactcaggcacctcgacgctgaccattacggttaatagcaagaaaaccaaagatctggtcttcacgaaagaaaacaccatcacggtgcagcaatatgacagcaatggtaccaaactggaaggctccgctgtggaaatcacgaaactggatgaaatctgtaatgctctgaaaggtactagtgacaaaaacaatggctctggtagcaaagagaaaaacaaagatggcaagtactcattcaacgaaaaaggcgaactgtcggcgaaaacgatgacgcgtgaaaacggcaccaaactggaatatacggaaatgaaaagcgatggcaccggtaaagcgaaagaagttctgaaaaactttaccctggaaggcaaagtcgccaatgacaaagtcaccctggaagtgaaatgcggcaccgttacgctgtcaaaagaaattgcaaaatcgggtgaagtgaccgttgctctgaacgatacgaataccacgcaagcgaccaagaaaaccggcgcctgggacagcaaaacctctacgctgaccattagtgttaatagcaagaaaaccacgcagctggtcttcaccaaacaagatacgatcaccgtgcagaaatacgacagtgcgggtaccaacctggaaggcacggctgttgaaatcaaaaccctggacgaactgtgtaacgccctgaaa

SEQ ID NO: 50 - protein, 320 aa, Artificial Sequence
  Artificial sequence
  LIPID (1)..(1)
CSSFNEKGEVSEKIITRADGTRLEYTGIKSDGSGKAKEVLKNFTLEGKVANDKTTLVVKCGTVTLSKNISKSGEVSVELNDTDSSAATKKTAAWNSGTSTLTITVNSKKTKDLVFTKENTITVQQYDSNGTKLEGSAVEITKLDEICNALKGTSDKNNGSGSKEKNKDGKYSFNEKGELSAKTMTRENGTKLEYTEMKSDGTGKAKEVLKNFTLEGKVANDKVTLEVKCGTVTLSKEIAKSGEVTVALNDTNTTQATKKTGAWDSKTSTLTISVNSKKTTQLVFTKQDTITVQKYDSAGTNLEGTAVEIKTLDELCNALK

SEQ ID NO: 51 - DNA, 1023 bp, Artificial Sequence
  Artificial sequence
atgaaagctactaaactggtactgggcgcggtaatcctgggttctactctgctggcaggttgctcaagcttcaatgctaagggcgaactgagcgaaaaaacgatcctgcgtgcgaatggcacccgtctggaatacaccgaaatcaaatccgatggtacgggcaaagcaaaggaagtcctgaaagattttgctctggaaggtaccctggcggccgacaaaaccacgctgaaggtgacgtgcggcaccgtggttctgagcaaacatattccgaactctggtgaaatcaccgttgaactgaacgatagcaattctacgcaggcaaccaaaaagacgggcaaatgggacagtaatacctccacgctgaccatttcagtcaactcgaaaaagaccaaaaatattgtgttcacgaaggaagatacgatcaccgttcaaaaatatgactccgcgggcaccaacctggaaggcaatgccgtcgaaatcaaaaccctggatgaactgtgtaacgccctgaagggtactagtgacaaaaacaatggctctggtagcaaagagaaaaacaaagatggcaagtactcatttaacgataagggcaaactgtcggaaaaagtggtcacccgcgcaaatggcacccgcctggaatacacggaaatcaaaaacgatggtagcggcaaagcgaaggaagttctgaaaggctttgccctggaaggtaccctgacggatggcggtgaaaccaaactgaccgtgacgtgcggcaccgttacgctgtctaaaaacattagcaagtctggtgaaatcacggtcgcactgaatgataccgaaaccacgccggctgacaaaaagaccggcgaatggaaaagtgacacctccacgctgaccatttcaaagaactcgcagaaaccgaagcaactggtcttcaccaaagaaaacacgatcaccgtgcagaactataatcgtgccggtaatgctctggaaggctcaccggctgaaatcaaggacctggctgaactgtgtgcggcactgaaa

SEQ ID NO: 52 - protein, 321 aa, Artificial Sequence
  Artificial sequence
  LIPID (1)..(1)
CSSFNAKGELSEKTILRANGTRLEYTEIKSDGTGKAKEVLKDFALEGTLAADKTTLKVTCGTVVLSKHIPNSGEITVELNDSNSTQATKKTGKWDSNTSTLTISVNSKKTKNIVFTKEDTITVQKYDSAGTNLEGNAVEIKTLDELCNALKGTSDKNNGSGSKEKNKDGKYSFNDKGKLSEKVVTRANGTRLEYTEIKNDGSGKAKEVLKGFALEGTLTDGGETKLTVTCGTVTLSKNISKSGEITVALNDTETTPADKKTGEWKSDTSTLTISKNSQKPKQLVFTKENTITVQNYNRAGNALEGSPAEIKDLAELCAALK

SEQ ID NO: 53 - DNA, 1023 bp, Artificial Sequence
  Artificial sequence
atgaaagctactaaactggtactgggcgcggtaatcctgggttctactctgctggcaggttgctcaagcttcaacgaaaagggcgaaatctcagaaaaaaccatcgtccgcgctaacggcacccgcctggaatacaccgacatcaaatcagacaagaccggtaaagcgaaggaagttctgaaagattttacgctggaaggtaccctggcagcagacggtaaaaccacgctgaaggtgacctgcggtaccgttacgctgtccaaaaacattagtaagtccggcgaaatcacggtcgccctggatgacaccgatagctctggcaacaaaaagagcggtacctgggattcaggcacctcgacgctgaccatttctaaaaatcgtacgaaaaccaagcagctggtcttcacgaaagaagatacgatcaccgtgcaaaactatgacagcgcaggtaccaatctggaaggcaaagctgtggaaattaccacgctgaaagaactgtgtaatgctctgaaaggtactagtgacaaaaacaatggctctggtagcaaagagaaaaacaaagatggcaagtactcattcaacggcaaaggtgaaacgagcgaaaagaccatcgtgcgtgcgaacggtacccgcctggaatatacggacattaaatcggacggcagcggcaaagcaaaggaagtcctgaaagattttacgctggaaggtaccctggcagcagacggtaaaaccacgctgaaggtgacgtgcggcaccgtggttctgtcaaaaaacattctgaagtcgggtgaaatcaccgcagctctggatgacagcgataccacgcgtgctacgaaaaagaccggtaaatgggatagcaagacctctacgctgaccattagtgtcaactcccagaaaacgaagaatctggtgttcaccaaagaagatacgatcaccgttcaacgctatgacagtgcgggcaccaacctggaaggcaaagccgttgaaattaccacgctgaaagaactgtgtaatgctctgaaa

SEQ ID NO: 54 - protein, 321 aa, Artificial Sequence
  Artificial sequence
  LIPID (1)..(1)
CSSFNEKGEISEKTIVRANGTRLEYTDIKSDKTGKAKEVLKDFTLEGTLAADGKTTLKVTCGTVTLSKNISKSGEITVALDDTDSSGNKKSGTWDSGTSTLTISKNRTKTKQLVFTKEDTITVQNYDSAGTNLEGKAVEITTLKELCNALKGTSDKNNGSGSKEKNKDGKYSFNGKGETSEKTIVRANGTRLEYTDIKSDGSGKAKEVLKDFTLEGTLAADGKTTLKVTCGTVVLSKNILKSGEITAALDDSDTTRATKKTGKWDSKTSTLTISVNSQKTKNLVFTKEDTITVQRYDSAGTNLEGKAVEITTLKELCNALK

SEQ ID NO: 55 - protein, 148 aa, Artificial Sequence
  Artificial sequence
FNEKGEVSEKIITRADGTRLEYTGIKSDGSGKAKEVLKNFTLEGKVANDKTTLVVKCGTVTLSKNISKSGEVSVELNDTDSSAATKKTAAWNSGTSTLTITVNSKKTKDLVFTKENTITVQQYDSNGTKLEGSAVEITKLDEICNALK

SEQ ID NO: 56 - protein, 148 aa, Artificial Sequence
  Artificial sequence
FNEKGELSAKTMTRENGTKLEYTEMKSDGTGKAKEVLKNFTLEGKVANDKVTLEVKCGTVTLSKEIAKSGEVTVALNDTNTTQATKKTGAWDSKTSTLTISVNSKKTTQLVFTKQDTITVQKYDSAGTNLEGTAVEIKTLDELCNALK

SEQ ID NO: 57 - protein, 149 aa, Artificial Sequence
  Artificial sequence
FNDKGKLSEKVVTRANGTRLEYTEIKNDGSGKAKEVLKGFALEGTLTDGGETKLTVTCGTVTLSKNISKSGEITVALNDTETTPADKKTGEWKSDTSTLTISKNSQKTKQLVFTKENTITVQNYNRAGNALEGSPAEIKDLAELCAALK

SEQ ID NO: 58 - protein, 148 aa, Artificial Sequence
  Artificial sequence
FNAKGELSEKTILRANGTRLEYTEIKSDGTGKAKEVLKDFALEGTLAADKTTLKVTCGTVVLSKHIPNSGEITVELNDSNSTQATKKTGKWDSNTSTLTISVNSKKTKNIVFTKEDTITVQKYDSAGTNLEGNAVEIKTLDELCNALK

SEQ ID NO: 59 - protein, 148 aa, Artificial Sequence
  Artificial sequence
FNEKGEISEKTIVRANGTRLEYTDIKSDKTGKAKEVLKDFTLEGTLAADGKTTLKVTCGTVTLSKNISKSGEITVALDDTDSSGNKKSGTWDSGTSTLTISKNRTKTKQLVFTKEDTITVQNYDSAGTNLEGKAVEITTLKELCNALK

SEQ ID NO: 60 - protein, 149 aa, Artificial Sequence
  Artificial sequence
FNGKGETSEKTIVRANGTRLEYTDIKSDGSGKAKEVLKDFTLEGTLAADGKTTLKVTCGTVVLSKNILKSGEITAALDDSDTTRATKKTGKWDSKTSTLTISVNSQKTKNLVFTKEDTITVQRYDSAGTNLEGKAVEITTLKELCNALK

SEQ ID NO: 61 - protein, 150 aa, Artificial Sequence; identical to SEQ ID NO: 41
  Artificial sequence

SEQ ID NO: 62 - protein, 150 aa, Artificial Sequence
  Artificial sequence
FNEKGEVSEKILTRSNGTTLEYSQMTDAENATKAVETLKNGIKLPGNLVGGKTTLKITCGTVTLSKHIAKSGEVTVEINDTSSTPNTKKTGKWDARNSTLTIIVDSKNKTKLVFTKQDTITVQSYNPAGNKLEGTAVEIKTLQELCNALK

SEQ ID NO: 63 - protein, 148 aa, Artificial Sequence
  Artificial sequence
FNEKGELSEKTLVRANGTKLEYTEIKSDGTGKAKEVLKDFTLEGTLANEKTKLTVTCGTVTLSKNISKSGEITVALNDTETTPADKKTGEWKSDTSTLTISKNSQKTKQLVFTKENTITVQNYNRAGNALEGSPAEIKDLAELCAALK

SEQ ID NO: 64 - protein, 148 aa, Artificial Sequence
  Artificial sequence
FNEKGELSEKTLVRANGTKLEYTEIKSDGTGKAKEVLKDFTLEGTLANEKATLTVKCGTVTLSKNIDKSGEVTVALNDTDSTAATKKTGAWDSKTSTLTITVNSKKTKDLVFTKQDTITVQKYDSAGTTLEGSAVEIKTLDELCNALK

SEQ ID NO: 65 - protein, 16 aa, Borrelia
MKKYLLGIGLILALIA

SEQ ID NO: 66 - protein, 15 aa, Borrelia
MRLLIGFALALALIG

SEQ ID NO: 67 - protein, 20 aa, Escherichia coli
MKATKLVLGAVILGSTLLAG

SEQ ID NO: 68 - protein, 21 aa, Artificial Sequence
  Artificial sequence
GTSDKNNGSGSKEKNKDGKYS

SEQ ID NO: 69 - protein, 278 aa, Artificial Sequence
  Artificial sequence
MRLLIGFALALALIGCAQKGAESIGSVSVDLPGEMKVLVSKEKDKNGKYDLIATVDKLELKGTSDKNNGSGVLEGVKTNKSKVKLTISDDLGQTTLEVFKEDGKTLVSKKVTSKDKSSTEEKFNEKGEVSEKIITMADGTRLEYTGIKSDGTGKAKYVLKNFTLEGKVANDKTTLEVKEGTVTLSMNISKSGEVSVELNDTDSSAATKKTAAWNSKTSTLTISVNSKKTTQLVFTKQDTITVQKYDSAGTNLEGTAVEIKTLDELKNALKLEHHHHHH

SEQ ID NO: 70 - protein, 278 aa, Artificial Sequence
  Artificial sequence
MRLLIGFALALALIGCAQKGAESIGSVSVDLPGGMKVLVSKEKDKNGKYSLMATVEKLELKGTSDKNNGSGTLEGEKTNKSKVKLTIAEDLSKTTFEIFKEDGKTLVSKKVTLKDKSSTEEKFNEKGEISEKTIVMANGTRLEYTDIKSDKTGKAKYVLKDFTLEGTLAADGKTTLKVTEGTVTLSMNISKSGEITVALDDTDSSGNKKSGTWDSDTSTLTISKNSQKTKQLVFTKENTITVQNYNRAGNALEGSPAEIKDLAELKAALKLEHHHHHH

SEQ ID NO: 71 - protein, 279 aa, Artificial Sequence
  Artificial sequence
MRLLIGFALALALIGCAQKGAESIGSVSVDLPGGMTVLVSKEKDKNGKYSLEATVDKLELKGTSDKNNGSGTLEGEKTNKSKVKLTIADDLSQTKFEIFKEDAKTLVSKKVTLKDKSSTEEKFNEKGETSEKTIVMANGTRLEYTDIKSDGSGKAKYVLKDFTLEGTLAADGKTTLKVTEGTVVLSMNILKSGEITVALDDSDTTQATKKTGKWDSNTSTLTISVNSKKTKNIVFTKEDTITVQKYDSAGTNLEGNAVEIKTLDELKNALKLEHHHHHH

SEQ ID NO: 72 - protein, 320 aa, Artificial Sequence
  Artificial sequence
  LIPID (1)..(1)
CSSFNAKGELSEKTILRANGTRLEYTEIKSDGTGKAKEVLKDFALEGTLAADKTTLKVTCGTVVLSKHIPNSGEITVELNDSNSTQATKKTGKWDSNTSTLTISVNSKKTKNIVFTKEDTITVQKYDSAGTNLEGNAVEIKTLDELCNALKGTSDKNNGSGSKEKNKDGKYSFNEKGELSEKTLVRANGTKLEYTEIKSDGTGKAKEVLKDFTLEGTLANEKTKLTVTCGTVTLSKNISKSGEITVALNDTETTPADKKTGEWKSDTSTLTISKNSQKTKQLVFTKENTITVQNYNRAGNALEGSPAEIKDLAELCAALK

SEQ ID NO: 73 - protein, 50 aa, Borrelia spielmanii
FNEKGELSEKTLVRANGTKLEYTEIKSDGTGKAKEVLKDFTLEGTLANEK

SEQ ID NO: 74 - protein, 273 aa, Borrelia afzelii
MKKYLLGIGLILALIACKQNVSSLDEKNSASVDLPGEMKVLVSKEKDKDGKYSLKATVDKIELKGTSDKDNGSGVLEGTKDDKSKAKLTIADDLSKTTFELFKEDGKTLVSRKVSSKDKTSTDEMFNEKGELSAKTMTRENGTKLEYTEMKSDGTGKAKEVLKNFTLEGKVANDKVTLEVKEGTVTLSKEIAKSGEVTVALNDTNTTQATKKTGAWDSKTSTLTISVNSKKTTQLVFTKQDTITVQKYDSAGTNLEGTAVEIKTLDELKNALK

SEQ ID NO: 75 - protein, 8 aa, Artificial Sequence
  Artificial sequence
LEHHHHHH